European Patent Specification EP 4 291 164 B1, published July 8, 2026. Title: ENGINEERED EXTRACELLULAR VESICLES AND THEIR USES. Applicant: Wake Forest University Health Sciences. The sequence listing filed with the application follows.

SEQUENCE LISTING (116 sequences)

SEQ ID NO: 1 - DNA, 351 bp, Artificial Sequence
  Synthetic construct
atggcttctaactttactcagttcgttctcgtcgacaatggcggaactggcgacgtgactgtcgccccaagcaacttcgctaacgggatcgctgaatggatcagctctaactcgcgttcacaggcttacaaagtaacctgtagcgttcgtcagagctctgcgcagaatcgcaaatacaccatcaaagtcgaggtgcctaaaggcgcctggcgttcgtacttaaatatggaactaaccattccaattttcgccacgaattccgactgcgagcttattgttaaggcaatgcaaggtctcctaaaagatggaaacccgattccctcagcaatcgcagcaaactccggcatctac

SEQ ID NO: 2 - protein, 117 aa, Artificial Sequence
  Synthetic construct
MASNFTQFVLVDNGGTGDVTVAPSNFANGIAEWISSNSRSQAYKVTCSVRQSSAQNRKYTIKVEVPKGAWRSYLNMELTIPIFATNSDCELIVKAMQGLLKDGNPIPSAIAANSGIY

SEQ ID NO: 3 - DNA, 363 bp, Artificial Sequence
  Synthetic construct
tccaaaacaatagtcctctccgtaggggaggcaacacggactttgaccgaaatccagtcaaccgctgaccgacaaatctttgaagagaaagtagggcctcttgtgggccgactgcgcttgactgcaagcttgcgacaaaacggcgcaaagactgcctatagggtcaaccttaaactcgaccaagccgacgtggtcgatagcggtctccctaaggttcggtatacgcaggtctggagtcatgacgtaacaatcgtagcaaacagcacagaagcctcccgaaaaagcctctacgatctgacgaaatccttggtggctacgtcacaggtggaagacctcgttgtcaaccttgtacctctgggtcga

SEQ ID NO: 4 - protein, 121 aa, Artificial Sequence
  Synthetic construct
SKTIVLSVGEATRTLTEIQSTADRQIFEEKVGPLVGRLRLTASLRQNGAKTAYRVNLKLDQADVVDSGLPKVRYTQVWSHDVTIVANSTEASRKSLYDLTKSLVATSQVEDLVVNLVPLGR

SEQ ID NO: 5 - DNA, 66 bp, Artificial Sequence
  Synthetic construct
atggatgcacaaacacgccgccgcgaacgtcgcgcagagaaacaggctcaatggaaagcagcaaat

SEQ ID NO: 6 - protein, 22 aa, Artificial Sequence
  Synthetic construct
MDAQTRRRERRAEKQAQWKAAN

SEQ ID NO: 7 - DNA, 193 bp, Artificial Sequence
  Synthetic construct
atgaaatcaattcgctgtaaaaactgcaacaaactgttatttaaggcggattcctttgatcacattgaaatcaggtgtccgcgttgcaaacgtcacatcataatgctgaatgcctgcgagcatcccacggagaaacattgtgggaaaagagaaaaaatcacgcattctgacgaaaccgtgcgttattgagtat

SEQ ID NO: 8 - protein, 62 aa, Artificial Sequence
  Synthetic construct
MKSIRCKNCNKLLFKADSFDHIEIRCPRCKRHIIMLNACEHPTEKHCGKREKITHSDETVRY

SEQ ID NO: 9 - DNA, 15 bp, Artificial Sequence
  Synthetic construct
acagaggacacccag

SEQ ID NO: 10 - DNA, 19 bp, Artificial Sequence
  Synthetic construct
acatgaggatcacccatgt

SEQ ID NO: 11 - DNA, 21 bp, Artificial Sequence
  Synthetic construct
ggagcagacgaaggcgcgccc

SEQ ID NO: 12 - DNA, 25 bp, Artificial Sequence
  Synthetic construct
ggagcagacgatatggcgtcgctcc

SEQ ID NO: 13 - DNA, 18 bp, Artificial Sequence
  Synthetic construct
gggcccgaagaagggccc

SEQ ID NO: 14 - DNA, 19 bp, Artificial Sequence
  Synthetic construct
gggccctgaagaagggccc

SEQ ID NO: 15 - DNA, 15 bp, Artificial Sequence
  Synthetic construct
cgaagccgcgagcac

SEQ ID NO: 16 - DNA, 18 bp, Artificial Sequence
  Synthetic construct
ctgaatgcctgcgagcat

SEQ ID NO: 17 - DNA, 132 bp, Artificial Sequence
  Synthetic construct
gctcgctttcttgctgtccaatttctattaaaggttcctttgttccctaagtccaactactaaactgggggatattatgaagggccttgagcatctggattctgcctaataaaaaacatttattttcattgc

SEQ ID NO: 18 - DNA, 84 bp, Artificial Sequence
  Synthetic construct
gccgccgcgccaacaaaaggccgcccaagccaacacaaacgggggaaagaagggccgagcacggacgccaaaaaaaacaacagc

SEQ ID NO: 19 - DNA, 5403 bp, Artificial Sequence
  Synthetic construct
atgaaacggacagccgacggaagcgagttcgagtcaccaaagaagaagcggaaagtctctgaagtcgagtttagccacgagtattggatgaggcacgcactgaccctggcaaagcgagcatgggatgaaagagaagtccccgtgggcgccgtgctggtgcacaacaatagagtgatcggagagggatggaacaggccaatcggccgccacgaccctaccgcacacgcagagatcatggcactgaggcagggaggcctggtcatgcagaattaccgcctgatcgatgccaccctgtatgtgacactggagccatgcgtgatgtgcgcaggagcaatgatccacagcaggatcggaagagtggtgttcggagcacgggacgccaagaccggcgcagcaggctccctgatggatgtgctgcaccaccccggcatgaaccaccgggtggagatcacagagggaatcctggcagacgagtgcgccgccctgctgagcgatttctttagaatgcggagacaggagatcaaggcccagaagaaggcacagagctccaccgactctggaggatctagcggaggatcctctggaagcgagacaccaggcacaagcgagtccgccacaccagagagctccggcggctcctccggaggatcctctgaggtggagttttcccacgagtactggatgagacatgccctgaccctggccaagagggcacgcgatgagagggaggtgcctgtgggagccgtgctggtgctgaacaatagagtgatcggcgagggctggaacagagccatcggcctgcacgacccaacagcccatgccgaaattatggccctgagacagggcggcctggtcatgcagaactacagactgattgacgccaccctgtacgtgacattcgagccttgcgtgatgtgcgccggcgccatgatccactctaggatcggccgcgtggtgtttggcgtgaggaacgcaaaaaccggcgccgcaggctccctgatggacgtgctgcactaccccggcatgaatcaccgcgtcgaaattaccgagggaatcctggcagatgaatgtgccgccctgctgtgctatttctttcggatgcctagacaggtgttcaatgctcagaagaaggcccagagctccaccgactccggaggatctagcggaggctcctctggctctgagacacctggcacaagcgagagcgcaacacctgaaagcagcgggggcagcagcggggggtcagacaagaagtacagcatcggcctggccatcggcaccaactctgtgggctgggccgtgatcaccgacgagtacaaggtgcccagcaagaaattcaaggtgctgggcaacaccgaccggcacagcatcaagaagaacctgatcggagccctgctgttcgacagcggcgaaacagccgaggccacccggctgaagagaaccgccagaagaagatacaccagacggaagaaccggatctgctatctgcaagagatcttcagcaacgagatggccaaggtggacgacagcttcttccacagactggaagagtccttcctggtggaagaggataagaagcacgagcggcaccccatcttcggcaacatcgtggacgaggtggcctaccacgagaagtaccccaccatctaccacctgagaaagaaactggtggacagcaccgacaaggccgacctgcggctgatctatctggccctggcccacatgatcaagttccggggccacttcctgatcgagggcgacctgaaccccgacaacagcgacgtggacaagctgttcatccagctggtgcagacctacaaccagctgttcgaggaaaaccccatcaacgccagcggcgtggacgccaaggccatcctgtctgccagactgagcaagagcagacggctggaaaatctgatcgcccagctgcccggcgagaagaagaatggcctgttcggaaacctgattgccctgagcctgggcctgacccccaacttcaagagcaacttcgacctggccgaggatgccaaactgcagctgagcaaggacacctacgacgacgacctggacaacctgctggcccagatcggcgaccagtacgccgacctgtttctggccgccaagaacctgtccgacgccatcctgctgagcgacatcctgagagtgaacaccgagatcaccaaggcccccctgagcgcctctatgatcaagagatacgacgagcaccaccaggacctgaccctgctgaaagctctcgtgcggcagcagctgcctgagaagtacaaagagattttcttcgaccagagcaagaacggctacgccggctacattgacggcggagccagccaggaagagttctacaagttcatcaagcccatcctggaaaagatggacggcaccgaggaactgctcgtgaagctgaacagagaggacctgctgcggaagcagcggaccttcgacaacggcagcatcccccaccagatccacctgggagagctgcacgccattctgcggcggcaggaagatttttacccattcctgaaggacaaccgggaaaagatcgagaagatcctgaccttccgcatcccctactacgtgggccctctggccaggggaaacagcagattcgcctggatgaccagaaagagcgaggaaaccatcaccccctggaacttcgaggaagtggtggacaagggcgcttccgcccagagcttcatcgagcggatgaccaacttcgataagaacctgcccaacgagaaggtgctgcccaagcacagcctgctgtacgagtacttcaccgtgtataacgagctgaccaaagtgaaatacgtgaccgagggaatgagaaagcccgccttcctgagcggcgagcagaaaaaggccatcgtggacctgctgttcaagaccaaccggaaagtgaccgtgaagcagctgaaagaggactacttcaagaaaatcgagtgcttcgactccgtggaaatctccggcgtggaagatcggttcaacgcctccctgggcacataccacgatctgctgaaaattatcaaggacaaggacttcctggacaatgaggaaaacgaggacattctggaagatatcgtgctgaccctgacactgtttgaggacagagagatgatcgaggaacggctgaaaacctatgcccacctgttcgacgacaaagtgatgaagcagctgaagcggcggagatacaccggctggggcaggctgagccggaagctgatcaacggcatccgggacaagcagtccggcaagacaatcctggatttcctgaagtccgacggcttcgccaacagaaacttcatgcagctgatccacgacgacagcctgacctttaaagaggacatccagaaagcccaggtgtccggccagggcgatagcctgcacgagcacattgccaatctggccggcagccccgccattaagaagggcatcctgcagacagtgaaggtggtggacgagctcgtgaaagtgatgggccggcacaagcccgagaacatcgtgatcgaaatggccagagagaaccagaccacccagaagggacagaagaacagccgcgagagaatgaagcggatcgaagagggcatcaaagagctgggcagccagatcctgaaagaacaccccgtggaaaacacccagctgcagaacgagaagctgtacctgtactacctgcagaatgggcgggatatgtacgtggaccaggaactggacatcaaccggctgtccgactacgatgtggaccatatcgtgcctcagagctttctgaaggacgactccatcgacaacaaggtgctgaccagaagcgacaagaaccggggcaagagcgacaacgtgccctccgaagaggtcgtgaagaagatgaagaactactggcggcagctgctgaacgccaagctgattacccagagaaagttcgacaatctgaccaaggccgagagaggcggcctgagcgaactggataaggccggcttcatcaagagacagctggtggaaacccggcagatcacaaagcacgtggcacagatcctggactcccggatgaacactaagtacgacgagaatgacaagctgatccgggaagtgaaagtgatcaccctgaagtccaagctggtgtccgatttccggaaggatttccagttttacaaagtgcgcgagatcaacaactaccaccacgcccacgacgcctacctgaacgccgtcgtgggaaccgccctgatcaaaaagtaccctaagctggaaagcgagttcgtgtacggcgactacaaggtgtacgacgtgcggaagatgatcgccaagagcgagcaggaaatcggcaaggctaccgccaagtacttcttctacagcaacatcatgaactttttcaagaccgagattaccctggccaacggcgagatccggaagcggcctctgatcgagacaaacggcgaaaccggggagatcgtgtgggataagggccgggattttgccaccgtgcggaaagtgctgagcatgccccaagtgaatatcgtgaaaaagaccgaggtgcagacaggcggcttcagcaaagagtctatcctgcccaagaggaacagcgataagctgatcgccagaaagaaggactgggaccctaagaagtacggcggcttcgacagccccaccgtggcctattctgtgctggtggtggccaaagtggaaaagggcaagtccaagaaactgaagagtgtgaaagagctgctggggatcaccatcatggaaagaagcagcttcgagaagaatcccatcgactttctggaagccaagggctacaaagaagtgaaaaaggacctgatcatcaagctgcctaagtactccctgttcgagctggaaaacggccggaagagaatgctggcctctgccggcgaactgcagaagggaaacgaactggccctgccctccaaatatgtgaacttcctgtacctggccagccactatgagaagctgaagggctcccccgaggataatgagcagaaacagctgtttgtggaacagcacaagcactacctggacgagatcatcgagcagatcagcgagttctccaagagagtgatcctggccgacgctaatctggacaaagtgctgtccgcctacaacaagcaccgggataagcccatcagagagcaggccgagaatatcatccacctgtttaccctgaccaatctgggagcccctgccgccttcaagtactttgacaccaccatcgaccggaagaggtacaccagcaccaaagaggtgctggacgccaccctgatccaccagagcatcaccggcctgtacgagacacggatcgacctgtctcagctgggaggcgacaaaaggccggcggccacgaaaaaggccggccaggcaaaaaagaaaaagggatcctaa

SEQ ID NO: 20 - protein, 1800 aa, Artificial Sequence
  Synthetic construct
MKRTADGSEFESPKKKRKVSEVEFSHEYWMRHALTLAKRAWDEREVPVGAVLVHNNRVIGEGWNRPIGRHDPTAHAEIMALRQGGLVMQNYRLIDATLYVTLEPCVMCAGAMIHSRIGRVVFGARDAKTGAAGSLMDVLHHPGMNHRVEITEGILADECAALLSDFFRMRRQEIKAQKKAQSSTDSGGSSGGSSGSETPGTSESATPESSGGSSGGSSEVEFSHEYWMRHALTLAKRARDEREVPVGAVLVLNNRVIGEGWNRAIGLHDPTAHAEIMALRQGGLVMQNYRLIDATLYVTFEPCVMCAGAMIHSRIGRVVFGVRNAKTGAAGSLMDVLHYPGMNHRVEITEGILADECAALLCYFFRMPRQVFNAQKKAQSSTDSGGSSGGSSGSETPGTSESATPESSGGSSGGSDKKYSIGLAIGTNSVGWAVITDEYKVPSKKFKVLGNTDRHSIKKNLIGALLFDSGETAEATRLKRTARRRYTRRKNRICYLQEIFSNEMAKVDDSFFHRLEESFLVEEDKKHERHPIFGNIVDEVAYHEKYPTIYHLRKKLVDSTDKADLRLIYLALAHMIKFRGHFLIEGDLNPDNSDVDKLFIQLVQTYNQLFEENPINASGVDAKAILSARLSKSRRLENLIAQLPGEKKNGLFGNLIALSLGLTPNFKSNFDLAEDAKLQLSKDTYDDDLDNLLAQIGDQYADLFLAAKNLSDAILLSDILRVNTEITKAPLSASMIKRYDEHHQDLTLLKALVRQQLPEKYKEIFFDQSKNGYAGYIDGGASQEEFYKFIKPILEKMDGTEELLVKLNREDLLRKQRTFDNGSIPHQIHLGELHAILRRQEDFYPFLKDNREKIEKILTFRIPYYVGPLARGNSRFAWMTRKSEETITPWNFEEVVDKGASAQSFIERMTNFDKNLPNEKVLPKHSLLYEYFTVYNELTKVKYVTEGMRKPAFLSGEQKKAIVDLLFKTNRKVTVKQLKEDYFKKIECFDSVEISGVEDRFNASLGTYHDLLKIIKDKDFLDNEENEDILEDIVLTLTLFEDREMIEERLKTYAHLFDDKVMKQLKRRRYTGWGRLSRKLINGIRDKQSGKTILDFLKSDGFANRNFMQLIHDDSLTFKEDIQKAQVSGQGDSLHEHIANLAGSPAIKKGILQTVKVVDELVKVMGRHKPENIVIEMARENQTTQKGQKNSRERMKRIEEGIKELGSQILKEHPVENTQLQNEKLYLYYLQNGRDMYVDQELDINRLSDYDVDHIVPQSFLKDDSIDNKVLTRSDKNRGKSDNVPSEEVVKKMKNYWRQLLNAKLITQRKFDNLTKAERGGLSELDKAGFIKRQLVETRQITKHVAQILDSRMNTKYDENDKLIREVKVITLKSKLVSDFRKDFQFYKVREINNYHHAHDAYLNAVVGTALIKKYPKLESEFVYGDYKVYDVRKMIAKSEQEIGKATAKYFFYSNIMNFFKTEITLANGEIRKRPLIETNGETGEIVWDKGRDFATVRKVLSMPQVNIVKKTEVQTGGFSKESILPKRNSDKLIARKKDWDPKKYGGFDSPTVAYSVLVVAKVEKGKSKKLKSVKELLGITIMERSSFEKNPIDFLEAKGYKEVKKDLIIKLPKYSLFELENGRKRMLASAGELQKGNELALPSKYVNFLYLASHYEKLKGSPEDNEQKQLFVEQHKHYLDEIIEQISEFSKRVILADANLDKVLSAYNKHRDKPIREQAENIIHLFTLTNLGAPAAFKYFDTTIDRKRYTSTKEVLDATLIHQSITGLYETRIDLSQLGGDKRPAATKKAGQAKKKKGS

SEQ ID NO: 21 - DNA, 4278 bp, Artificial Sequence
  Synthetic construct
atggactataaggaccacgacggagactacaaggatcatgatattgattacaaagacgatgacgataagatggccccaaagaagaagcggaaggtcggtatccacggagtcccagcagccgacaagaagtacagcatcggcctggacatcggcaccaactctgtgggctgggccgtgatcaccgacgagtacaaggtgcccagcaagaaattcaaggtgctgggcaacaccgaccggcacagcatcaagaagaacctgatcggagccctgctgttcgacagcggcgaaacagccgaggccacccggctgaagagaaccgccagaagaagatacaccagacggaagaaccggatctgctatctgcaagagatcttcagcaacgagatggccaaggtggacgacagcttcttccacagactggaagagtccttcctggtggaagaggataagaagcacgagcggcaccccatcttcggcaacatcgtggacgaggtggcctaccacgagaagtaccccaccatctaccacctgagaaagaaactggtggacagcaccgacaaggccgacctgcggctgatctatctggccctggcccacatgatcaagttccggggccacttcctgatcgagggcgacctgaaccccgacaacagcgacgtggacaagctgttcatccagctggtgcagacctacaaccagctgttcgaggaaaaccccatcaacgccagcggcgtggacgccaaggccatcctgtctgccagactgagcaagagcagacggctggaaaatctgatcgcccagctgcccggcgagaagaagaatggcctgttcggaaacctgattgccctgagcctgggcctgacccccaacttcaagagcaacttcgacctggccgaggatgccaaactgcagctgagcaaggacacctacgacgacgacctggacaacctgctggcccagatcggcgaccagtacgccgacctgtttctggccgccaagaacctgtccgacgccatcctgctgagcgacatcctgagagtgaacaccgagatcaccaaggcccccctgagcgcctctatgatcaagagatacgacgagcaccaccaggacctgaccctgctgaaagctctcgtgcggcagcagctgcctgagaagtacaaagagattttcttcgaccagagcaagaacggctacgccggctacattgacggcggagccagccaggaagagttctacaagttcatcaagcccatcctggaaaagatggacggcaccgaggaactgctcgtgaagctgaacagagaggacctgctgcggaagcagcggaccttcgacaacggcagcatcccccaccagatccacctgggagagctgcacgccattctgcggcggcaggaagatttttacccattcctgaaggacaaccgggaaaagatcgagaagatcctgaccttccgcatcccctactacgtgggccctctggccaggggaaacagcagattcgcctggatgaccagaaagagcgaggaaaccatcaccccctggaacttcgaggaagtggtggacaagggcgcttccgcccagagcttcatcgagcggatgaccaacttcgataagaacctgcccaacgagaaggtgctgcccaagcacagcctgctgtacgagtacttcaccgtgtataacgagctgaccaaagtgaaatacgtgaccgagggaatgagaaagcccgccttcctgagcggcgagcagaaaaaggccatcgtggacctgctgttcaagaccaaccggaaagtgaccgtgaagcagctgaaagaggactacttcaagaaaatcgagtgcttcgactccgtggaaatctccggcgtggaagatcggttcaacgcctccctgggcacataccacgatctgctgaaaattatcaaggacaaggacttcctggacaatgaggaaaacgaggacattctggaagatatcgtgctgaccctgacactgtttgaggacagagagatgatcgaggaacggctgaaaacctatgcccacctgttcgacgacaaagtgatgaagcagctgaagcggcggagatacaccggctggggcaggctgagccggaagctgatcaacggcatccgggacaagcagtccggcaagacaatcctggatttcctgaagtccgacggcttcgccaacagaaacttcatgcagctgatccacgacgacagcctgacctttaaagaggacatccagaaagcccaggtgtccggccagggcgatagcctgcacgagcacattgccaatctggccggcagccccgccattaagaagggcatcctgcagacagtgaaggtggtggacgagctcgtgaaagtgatgggccggcacaagcccgagaacatcgtgatcgaaatggccagagagaaccagaccacccagaagggacagaagaacagccgcgagagaatgaagcggatcgaagagggcatcaaagagctgggcagccagatcctgaaagaacaccccgtggaaaacacccagctgcagaacgagaagctgtacctgtactacctgcagaatgggcgggatatgtacgtggaccaggaactggacatcaaccggctgtccgactacgatgtggaccatatcgtgcctcagagctttctgaaggacgactccatcgacaacaaggtgctgaccagaagcgacaagaaccggggcaagagcgacaacgtgccctccgaagaggtcgtgaagaagatgaagaactactggcggcagctgctgaacgccaagctgattacccagagaaagttcgacaatctgaccaaggccgagagaggcggcctgagcgaactggataaggccggcttcatcaagagacagctggtggaaacccggcagatcacaaagcacgtggcacagatcctggactcccggatgaacactaagtacgacgagaatgacaagctgatccgggaagtgaaagtgatcaccctgaagtccaagctggtgtccgatttccggaaggatttccagttttacaaagtgcgcgagatcaacaactaccaccacgcccacgacgcctacctgaacgccgtcgtgggaaccgccctgatcaaaaagtaccctaagctggaaagcgagttcgtgtacggcgactacaaggtgtacgacgtgcggaagatgatcgccaagagcgagcaggaaatcggcaaggctaccgccaagtacttcttctacagcaacatcatgaactttttcaagaccgagattaccctggccaacggcgagatccggaagcggcctctgatcgagacaaacggcgaaaccggggagatcgtgtgggataagggccgggattttgccaccgtgcggaaagtgctgagcatgccccaagtgaatatcgtgaaaaagaccgaggtgcagacaggcggcttcagcaaagagtctatcctgcccaagaggaacagcgataagctgatcgccagaaagaaggactgggaccctaagaagtacggcggcttcgacagccccaccgtggcctattctgtgctggtggtggccaaagtggaaaagggcaagtccaagaaactgaagagtgtgaaagagctgctggggatcaccatcatggaaagaagcagcttcgagaagaatcccatcgactttctggaagccaagggctacaaagaagtgaaaaaggacctgatcatcaagctgcctaagtactccctgttcgagctggaaaacggccggaagagaatgctggcctctgccggcgaactgcagaagggaaacgaactggccctgccctccaaatatgtgaacttcctgtacctggccagccactatgagaagctgaagggctcccccgaggataatgagcagaaacagctgtttgtggaacagcacaagcactacctggacgagatcatcgagcagatcagcgagttctccaagagagtgatcctggccgacgctaatctggacaaagtgctgtccgcctacaacaagcaccgggataagcccatcagagagcaggccgagaatatcatccacctgtttaccctgaccaatctgggagcccctgccgccttcaagtactttgacaccaccatcgaccggaagaggtacaccagcaccaaagaggtgctggacgccaccctgatccaccagagcatcaccggcctgtacgagacacggatcgacctgtctcagctgggaggcgacaaaaggccggcggccacgaaaaaggccggccaggcaaaaaagaaaaagggatcctaa

SEQ ID NO: 22 - protein, 1367 aa, Artificial Sequence
  Synthetic construct
DKKYSIGLAIGTNSVGWAVITDEYKVPSKKFKVLGNTDRHSIKKNLIGALLFDSGETAEATRLKRTARRRYTRRKNRICYLQEIFSNEMAKVDDSFFHRLEESFLVEEDKKHERHPIFGNIVDEVAYHEKYPTIYHLRKKLVDSTDKADLRLIYLALAHMIKFRGHFLIEGDLNPDNSDVDKLFIQLVQTYNQLFEENPINASGVDAKAILSARLSKSRRLENLIAQLPGEKKNGLFGNLIALSLGLTPNFKSNFDLAEDAKLQLSKDTYDDDLDNLLAQIGDQYADLFLAAKNLSDAILLSDILRVNTEITKAPLSASMIKRYDEHHQDLTLLKALVRQQLPEKYKEIFFDQSKNGYAGYIDGGASQEEFYKFIKPILEKMDGTEELLVKLNREDLLRKQRTFDNGSIPHQIHLGELHAILRRQEDFYPFLKDNREKIEKILTFRIPYYVGPLARGNSRFAWMTRKSEETITPWNFEEVVDKGASAQSFIERMTNFDKNLPNEKVLPKHSLLYEYFTVYNELTKVKYVTEGMRKPAFLSGEQKKAIVDLLFKTNRKVTVKQLKEDYFKKIECFDSVEISGVEDRFNASLGTYHDLLKIIKDKDFLDNEENEDILEDIVLTLTLFEDREMIEERLKTYAHLFDDKVMKQLKRRRYTGWGRLSRKLINGIRDKQSGKTILDFLKSDGFANRNFMQLIHDDSLTFKEDIQKAQVSGQGDSLHEHIANLAGSPAIKKGILQTVKVVDELVKVMGRHKPENIVIEMARENQTTQKGQKNSRERMKRIEEGIKELGSQILKEHPVENTQLQNEKLYLYYLQNGRDMYVDQELDINRLSDYDVDHIVPQSFLKDDSIDNKVLTRSDKNRGKSDNVPSEEVVKKMKNYWRQLLNAKLITQRKFDNLTKAERGGLSELDKAGFIKRQLVETRQITKHVAQILDSRMNTKYDENDKLIREVKVITLKSKLVSDFRKDFQFYKVREINNYHHAHDAYLNAVVGTALIKKYPKLESEFVYGDYKVYDVRKMIAKSEQEIGKATAKYFFYSNIMNFFKTEITLANGEIRKRPLIETNGETGEIVWDKGRDFATVRKVLSMPQVNIVKKTEVQTGGFSKESILPKRNSDKLIARKKDWDPKKYGGFDSPTVAYSVLVVAKVEKGKSKKLKSVKELLGITIMERSSFEKNPIDFLEAKGYKEVKKDLIIKLPKYSLFELENGRKRMLASAGELQKGNELALPSKYVNFLYLASHYEKLKGSPEDNEQKQLFVEQHKHYLDEIIEQISEFSKRVILADANLDKVLSAYNKHRDKPIREQAENIIHLFTLTNLGAPAAFKYFDTTIDRKRYTSTKEVLDATLIHQSITGLYETRIDLSQLGGD

SEQ ID NO: 23 - DNA, 4272 bp, Artificial Sequence
  Synthetic construct
atggactataaggaccacgacggagactacaaggatcatgatattgattacaaagacgatgacgataagatggccccaaagaagaagcggaaggtcggtatccacggagtcccagcagccgacaagaagtacagcatcggcctggacatcggcaccaactctgtgggctgggccgtgatcaccgacgagtacaaggtgcccagcaagaaattcaaggtgctgggcaacaccgaccggcacagcatcaagaagaacctgatcggagccctgctgttcgacagcggcgaaacagccgaggccacccggctgaagagaaccgccagaagaagatacaccagacggaagaaccggatctgctatctgcaagagatcttcagcaacgagatggccaaggtggacgacagcttcttccacagactggaagagtccttcctggtggaagaggataagaagcacgagcggcaccccatcttcggcaacatcgtggacgaggtggcctaccacgagaagtaccccaccatctaccacctgagaaagaaactggtggacagcaccgacaaggccgacctgcggctgatctatctggccctggcccacatgatcaagttccggggccacttcctgatcgagggcgacctgaaccccgacaacagcgacgtggacaagctgttcatccagctggtgcagacctacaaccagctgttcgaggaaaaccccatcaacgccagcggcgtggacgccaaggccatcctgtctgccagactgagcaagagcagacggctggaaaatctgatcgcccagctgcccggcgagaagaagaatggcctgttcggaaacctgattgccctgagcctgggcctgacccccaacttcaagagcaacttcgacctggccgaggatgccaaactgcagctgagcaaggacacctacgacgacgacctggacaacctgctggcccagatcggcgaccagtacgccgacctgtttctggccgccaagaacctgtccgacgccatcctgctgagcgacatcctgagagtgaacaccgagatcaccaaggcccccctgagcgcctctatgatcaagagatacgacgagcaccaccaggacctgaccctgctgaaagctctcgtgcggcagcagctgcctgagaagtacaaagagattttcttcgaccagagcaagaacggctacgccggctacattgacggcggagccagccaggaagagttctacaagttcatcaagcccatcctggaaaagatggacggcaccgaggaactgctcgtgaagctgaacagagaggacctgctgcggaagcagcggaccttcgacaacggcagcatcccccaccagatccacctgggagagctgcacgccattctgcggcggcaggaagatttttacccattcctgaaggacaaccgggaaaagatcgagaagatcctgaccttccgcatcccctactacgtgggccctctggccaggggaaacagcagattcgcctggatgaccagaaagagcgaggaaaccatcaccccctggaacttcgaggaagtggtggacaagggcgcttccgcccagagcttcatcgagcggatgaccaacttcgataagaacctgcccaacgagaaggtgctgcccaagcacagcctgctgtacgagtacttcaccgtgtataacgagctgaccaaagtgaaatacgtgaccgagggaatgagaaagcccgccttcctgagcggcgagcagaaaaaggccatcgtggacctgctgttcaagaccaaccggaaagtgaccgtgaagcagctgaaagaggactacttcaagaaaatcgagtgcttcgactccgtggaaatctccggcgtggaagatcggttcaacgcctccctgggcacataccacgatctgctgaaaattatcaaggacaaggacttcctggacaatgaggaaaacgaggacattctggaagatatcgtgctgaccctgacactgtttgaggacagagagatgatcgaggaacggctgaaaacctatgcccacctgttcgacgacaaagtgatgaagcagctgaagcggcggagatacaccggctggggcaggctgagccggaagctgatcaacggcatccgggacaagcagtccggcaagacaatcctggatttcctgaagtccgacggcttcgccaacagaaacttcatgcagctgatccacgacgacagcctgacctttaaagaggacatccagaaagcccaggtgtccggccagggcgatagcctgcacgagcacattgccaatctggccggcagccccgccattaagaagggcatcctgcagacagtgaaggtggtggacgagctcgtgaaagtgatgggccggcacaagcccgagaacatcgtgatcgaaatggccagagagaaccagaccacccagaagggacagaagaacagccgcgagagaatgaagcggatcgaagagggcatcaaagagctgggcagccagatcctgaaagaacaccccgtggaaaacacccagctgcagaacgagaagctgtacctgtactacctgcagaatgggcgggatatgtacgtggaccaggaactggacatcaaccggctgtccgactacgatgtggaccatatcgtgcctcagagctttctgaaggacgactccatcgacaacaaggtgctgaccagaagcgacaagaaccggggcaagagcgacaacgtgccctccgaagaggtcgtgaagaagatgaagaactactggcggcagctgctgaacgccaagctgattacccagagaaagttcgacaatctgaccaaggccgagagaggcggcctgagcgaactggataaggccggcttcatcaagagacagctggtggaaacccggcagatcacaaagcacgtggcacagatcctggactcccggatgaacactaagtacgacgagaatgacaagctgatccgggaagtgaaagtgatcaccctgaagtccaagctggtgtccgatttccggaaggatttccagttttacaaagtgcgcgagatcaacaactaccaccacgcccacgacgcctacctgaacgccgtcgtgggaaccgccctgatcaaaaagtaccctaagctggaaagcgagttcgtgtacggcgactacaaggtgtacgacgtgcggaagatgatcgccaagagcgagcaggaaatcggcaaggctaccgccaagtacttcttctacagcaacatcatgaactttttcaagaccgagattaccctggccaacggcgagatccggaagcggcctctgatcgagacaaacggcgaaaccggggagatcgtgtgggataagggccgggattttgccaccgtgcggaaagtgctgagcatgccccaagtgaatatcgtgaaaaagaccgaggtgcagacaggcggcttcagcaaagagtctatcctgcccaagaggaacagcgataagctgatcgccagaaagaaggactgggaccctaagaagtacggcggcttcgacagccccaccgtggcctattctgtgctggtggtggccaaagtggaaaagggcaagtccaagaaactgaagagtgtgaaagagctgctggggatcaccatcatggaaagaagcagcttcgagaagaatcccatcgactttctggaagccaagggctacaaagaagtgaaaaaggacctgatcatcaagctgcctaagtactccctgttcgagctggaaaacggccggaagagaatgctggcctctgccggcgaactgcagaagggaaacgaactggccctgccctccaaatatgtgaacttcctgtacctggccagccactatgagaagctgaagggctcccccgaggataatgagcagaaacagctgtttgtggaacagcacaagcactacctggacgagatcatcgagcagatcagcgagttctccaagagagtgatcctggccgacgctaatctggacaaagtgctgtccgcctacaacaagcaccgggataagcccatcagagagcaggccgagaatatcatccacctgtttaccctgaccaatctgggagcccctgccgccttcaagtactttgacaccaccatcgaccggaagaggtacaccagcaccaaagaggtgctggacgccaccctgatccaccagagcatcaccggcctgtacgagacacggatcgacctgtctcagctgggaggcgacaaaaggccggcggccacgaaaaaggccggccaggcaaaaaagaaaaagtaa

SEQ ID NO: 24 - protein, 1423 aa, Artificial Sequence
  Synthetic construct
MDYKDHDGDYKDHDIDYKDDDDKMAPKKKRKVGIHGVPAADKKYSIGLDIGTNSVGWAVITDEYKVPSKKFKVLGNTDRHSIKKNLIGALLFDSGETAEATRLKRTARRRYTRRKNRICYLQEIFSNEMAKVDDSFFHRLEESFLVEEDKKHERHPIFGNIVDEVAYHEKYPTIYHLRKKLVDSTDKADLRLIYLALAHMIKFRGHFLIEGDLNPDNSDVDKLFIQLVQTYNQLFEENPINASGVDAKAILSARLSKSRRLENLIAQLPGEKKNGLFGNLIALSLGLTPNFKSNFDLAEDAKLQLSKDTYDDDLDNLLAQIGDQYADLFLAAKNLSDAILLSDILRVNTEITKAPLSASMIKRYDEHHQDLTLLKALVRQQLPEKYKEIFFDQSKNGYAGYIDGGASQEEFYKFIKPILEKMDGTEELLVKLNREDLLRKQRTFDNGSIPHQIHLGELHAILRRQEDFYPFLKDNREKIEKILTFRIPYYVGPLARGNSRFAWMTRKSEETITPWNFEEVVDKGASAQSFIERMTNFDKNLPNEKVLPKHSLLYEYFTVYNELTKVKYVTEGMRKPAFLSGEQKKAIVDLLFKTNRKVTVKQLKEDYFKKIECFDSVEISGVEDRFNASLGTYHDLLKIIKDKDFLDNEENEDILEDIVLTLTLFEDREMIEERLKTYAHLFDDKVMKQLKRRRYTGWGRLSRKLINGIRDKQSGKTILDFLKSDGFANRNFMQLIHDDSLTFKEDIQKAQVSGQGDSLHEHIANLAGSPAIKKGILQTVKVVDELVKVMGRHKPENIVIEMARENQTTQKGQKNSRERMKRIEEGIKELGSQILKEHPVENTQLQNEKLYLYYLQNGRDMYVDQELDINRLSDYDVDHIVPQSFLKDDSIDNKVLTRSDKNRGKSDNVPSEEVVKKMKNYWRQLLNAKLITQRKFDNLTKAERGGLSELDKAGFIKRQLVETRQITKHVAQILDSRMNTKYDENDKLIREVKVITLKSKLVSDFRKDFQFYKVREINNYHHAHDAYLNAVVGTALIKKYPKLESEFVYGDYKVYDVRKMIAKSEQEIGKATAKYFFYSNIMNFFKTEITLANGEIRKRPLIETNGETGEIVWDKGRDFATVRKVLSMPQVNIVKKTEVQTGGFSKESILPKRNSDKLIARKKDWDPKKYGGFDSPTVAYSVLVVAKVEKGKSKKLKSVKELLGITIMERSSFEKNPIDFLEAKGYKEVKKDLIIKLPKYSLFELENGRKRMLASAGELQKGNELALPSKYVNFLYLASHYEKLKGSPEDNEQKQLFVEQHKHYLDEIIEQISEFSKRVILADANLDKVLSAYNKHRDKPIREQAENIIHLFTLTNLGAPAAFKYFDTTIDRKRYTSTKEVLDATLIHQSITGLYETRIDLSQLGGDKRPAATKKAGQAKKKK

SEQ ID NO: 25 - DNA, 3345 bp, Artificial Sequence
  Synthetic construct
atggccccaaagaagaagcggaaggtcggtatccacggagtcccagcagccaagcggaactacatcctgggcctggacatcggcatcaccagcgtgggctacggcatcatcgactacgagacacgggacgtgatcgatgccggcgtgcggctgttcaaagaggccaacgtggaaaacaacgagggcaggcggagcaagagaggcgccagaaggctgaagcggcggaggcggcatagaatccagagagtgaagaagctgctgttcgactacaacctgctgaccgaccacagcgagctgagcggcatcaacccctacgaggccagagtgaagggcctgagccagaagctgagcgaggaagagttctctgccgccctgctgcacctggccaagagaagaggcgtgcacaacgtgaacgaggtggaagaggacaccggcaacgagctgtccaccaaagagcagatcagccggaacagcaaggccctggaagagaaatacgtggccgaactgcagctggaacggctgaagaaagacggcgaagtgcggggcagcatcaacagattcaagaccagcgactacgtgaaagaagccaaacagctgctgaaggtgcagaaggcctaccaccagctggaccagagcttcatcgacacctacatcgacctgctggaaacccggcggacctactatgagggacctggcgagggcagccccttcggctggaaggacatcaaagaatggtacgagatgctgatgggccactgcacctacttccccgaggaactgcggagcgtgaagtacgcctacaacgccgacctgtacaacgccctgaacgacctgaacaatctcgtgatcaccagggacgagaacgagaagctggaatattacgagaagttccagatcatcgagaacgtgttcaagcagaagaagaagcccaccctgaagcagatcgccaaagaaatcctcgtgaacgaagaggatattaagggctacagagtgaccagcaccggcaagcccgagttcaccaacctgaaggtgtaccacgacatcaaggacattaccgcccggaaagagattattgagaacgccgagctgctggatcagattgccaagatcctgaccatctaccagagcagcgaggacatccaggaagaactgaccaatctgaactccgagctgacccaggaagagatcgagcagatctctaatctgaagggctataccggcacccacaacctgagcctgaaggccatcaacctgatcctggacgagctgtggcacaccaacgacaaccagatcgctatcttcaaccggctgaagctggtgcccaagaaggtggacctgtcccagcagaaagagatccccaccaccctggtggacgacttcatcctgagccccgtcgtgaagagaagcttcatccagagcatcaaagtgatcaacgccatcatcaagaagtacggcctgcccaacgacatcattatcgagctggcccgcgagaagaactccaaggacgcccagaaaatgatcaacgagatgcagaagcggaaccggcagaccaacgagcggatcgaggaaatcatccggaccaccggcaaagagaacgccaagtacctgatcgagaagatcaagctgcacgacatgcaggaaggcaagtgcctgtacagcctggaagccatccctctggaagatctgctgaacaaccccttcaactatgaggtggaccacatcatccccagaagcgtgtccttcgacaacagcttcaacaacaaggtgctcgtgaagcaggaagaaaacagcaagaagggcaaccggaccccattccagtacctgagcagcagcgacagcaagatcagctacgaaaccttcaagaagcacatcctgaatctggccaagggcaagggcagaatcagcaagaccaagaaagagtatctgctggaagaacgggacatcaacaggttctccgtgcagaaagacttcatcaaccggaacctggtggataccagatacgccaccagaggcctgatgaacctgctgcggagctacttcagagtgaacaacctggacgtgaaagtgaagtccatcaatggcggcttcaccagctttctgcggcggaagtggaagtttaagaaagagcggaacaaggggtacaagcaccacgccgaggacgccctgatcattgccaacgccgatttcatcttcaaagagtggaagaaactggacaaggccaaaaaagtgatggaaaaccagatgttcgaggaaaagcaggccgagagcatgcccgagatcgaaaccgagcaggagtacaaagagatcttcatcaccccccaccagatcaagcacattaaggacttcaaggactacaagtacagccaccgggtggacaagaagcctaatagagagctgattaacgacaccctgtactccacccggaaggacgacaagggcaacaccctgatcgtgaacaatctgaacggcctgtacgacaaggacaatgacaagctgaaaaagctgatcaacaagagccccgaaaagctgctgatgtaccaccacgacccccagacctaccagaaactgaagctgattatggaacagtacggcgacgagaagaatcccctgtacaagtactacgaggaaaccgggaactacctgaccaagtactccaaaaaggacaacggccccgtgatcaagaagattaagtattacggcaacaaactgaacgcccatctggacatcaccgacgactaccccaacagcagaaacaaggtcgtgaagctgtccctgaagccctacagattcgacgtgtacctggacaatggcgtgtacaagttcgtgaccgtgaagaatctggatgtgatcaaaaaagaaaactactacgaagtgaatagcaagtgctatgaggaagctaagaagctgaagaagatcagcaaccaggccgagtttatcgcctccttctacaacaacgatctgatcaagatcaacggcgagctgtatagagtgatcggcgtgaacaacgacctgctgaaccggatcgaagtgaacatgatcgacatcacctaccgcgagtacctggaaaacatgaacgacaagaggccccccaggatcattaagacaatcgcctccaagacccagagcattaagaagtacagcacagacattctgggcaacctgtatgaagtgaaatctaagaagcaccctcagatcatcaaaaagggcaaaaggccggcggccacgaaaaaggccggccaggcaaaaaagaaaaagggatcctacccatacgatgttccagattacgcttacccatacgatgttccagattacgcttacccatacgatgttccagattacgcttaa

SEQ ID NO: 26 - protein, 1114 aa, Artificial Sequence
  Synthetic construct
MAPKKKRKVGIHGVPAAKRNYILGLDIGITSVGYGIIDYETRDVIDAGVRLFKEANVENNEGRRSKRGARRLKRRRRHRIQRVKKLLFDYNLLTDHSELSGINPYEARVKGLSQKLSEEEFSAALLHLAKRRGVHNVNEVEEDTGNELSTKEQISRNSKALEEKYVAELQLERLKKDGEVRGSINRFKTSDYVKEAKQLLKVQKAYHQLDQSFIDTYIDLLETRRTYYEGPGEGSPFGWKDIKEWYEMLMGHCTYFPEELRSVKYAYNADLYNALNDLNNLVITRDENEKLEYYEKFQIIENVFKQKKKPTLKQIAKEILVNEEDIKGYRVTSTGKPEFTNLKVYHDIKDITARKEIIENAELLDQIAKILTIYQSSEDIQEELTNLNSELTQEEIEQISNLKGYTGTHNLSLKAINLILDELWHTNDNQIAIFNRLKLVPKKVDLSQQKEIPTTLVDDFILSPVVKRSFIQSIKVINAIIKKYGLPNDIIIELAREKNSKDAQKMINEMQKRNRQTNERIEEIIRTTGKENAKYLIEKIKLHDMQEGKCLYSLEAIPLEDLLNNPFNYEVDHIIPRSVSFDNSFNNKVLVKQEENSKKGNRTPFQYLSSSDSKISYETFKKHILNLAKGKGRISKTKKEYLLEERDINRFSVQKDFINRNLVDTRYATRGLMNLLRSYFRVNNLDVKVKSINGGFTSFLRRKWKFKKERNKGYKHHAEDALIIANADFIFKEWKKLDKAKKVMENQMFEEKQAESMPEIETEQEYKEIFITPHQIKHIKDFKDYKYSHRVDKKPNRELINDTLYSTRKDDKGNTLIVNNLNGLYDKDNDKLKKLINKSPEKLLMYHHDPQTYQKLKLIMEQYGDEKNPLYKYYEETGNYLTKYSKKDNGPVIKKIKYYGNKLNAHLDITDDYPNSRNKVVKLSLKPYRFDVYLDNGVYKFVTVKNLDVIKKENYYEVNSKCYEEAKKLKKISNQAEFIASFYNNDLIKINGELYRVIGVNNDLLNRIEVNMIDITYREYLENMNDKRPPRIIKTIASKTQSIKKYSTDILGNLYEVKSKKHPQIIKKGKRPAATKKAGQAKKKKGSYPYDVPDYAYPYDVPDYAYPYDVPDYA

SEQ ID NO: 27 - DNA, 119 bp, Artificial Sequence
  Synthetic construct
gcgcttgctcttcattccctgtttgagagctagaaatagcaagttcaaataaggctagtccgttatcaacttggctgaatgcctgcgagcatcccacccaagtggcaccgagtcggtgc

SEQ ID NO: 28 - DNA, 119 bp, Artificial Sequence
  Synthetic construct
gtaacggcagacttctcctcgtttgagagctagaaatagcaagttcaaataaggctagtccgttatcaacttggctgaatgcctgcgagcatcccacccaagtggcaccgagtcggtgc

SEQ ID NO: 29 - DNA, 119 bp, Artificial Sequence
  Synthetic construct
actgttgcctccggttctgagtttgagagctagaaatagcaagttcaaataaggctagtccgttatcaacttggctgaatgcctgcgagcatcccacccaagtggcaccgagtcggtgc

SEQ ID NO: 30 - DNA, 119 bp, Artificial Sequence
  Synthetic construct
gaggacaagtcgtacaatgggtttgagagctagaaatagcaagttcaaataaggctagtccgttatcaacttggctgaatgcctgcgagcatcccacccaagtggcaccgagtcggtgc

SEQ ID NO: 31 - DNA, 119 bp, Artificial Sequence
  Synthetic construct
ccattgttcaatatcgtccggtttgagagctagaaatagcaagttcaaataaggctagtccgttatcaacttggctgaatgcctgcgagcatcccacccaagtggcaccgagtcggtgc

SEQ ID NO: 32 - DNA, 119 bp, Artificial Sequence
  Synthetic construct
agccccagcaagagcacaaggtttgagagctagaaatagcaagttcaaataaggctagtccgttatcaacttggctgaatgcctgcgagcatcccacccaagtggcaccgagtcggtgc

SEQ ID NO: 33 - DNA, 119 bp, Artificial Sequence
  Synthetic construct
gatgagataatgatgagtcagtttgagagctagaaatagcaagttcaaataaggctagtccgttatcaacttggctgaatgcctgcgagcatcccacccaagtggcaccgagtcggtgc

SEQ ID NO: 34 - DNA, 117 bp, Artificial Sequence
  Synthetic construct
tatgtggctttaccaaggtccgtttaagtactctgctgaatgcctgcgagcatcccaccagaatctacttaaacaaggcaaaatgccgtgtttatctcgtcaacttgttggcgagat

SEQ ID NO: 35 - DNA, 116 bp, Artificial Sequence
  Synthetic construct
acacagacagactacacccagtttaagtactctgctgaatgcctgcgagcatcccaccagaatctacttaaacaaggcaaaatgccgtgtttatctcgtcaacttgttggcgagat

SEQ ID NO: 36 - DNA, 508 bp, Artificial Sequence
  Synthetic construct
cgttacataacttacggtaaatggcccgcctggctgaccgcccaacgacccccgcccattgacgtcaataatgacgtatgttcccatagtaacgccaatagggactttccattgacgtcaatgggtggagtatttacggtaaactgcccacttggcagtacatcaagtgtatcatatgccaagtacgccccctattgacgtcaatgacggtaaatggcccgcctggcattatgcccagtacatgaccttatgggactttcctacttggcagtacatctacgtattagtcatcgctattaccatggtgatgcggttttggcagtacatcaatgggcgtggatagcggtttgactcacggggatttccaagtctccaccccattgacgtcaatgggagtttgttttggcaccaaaatcaacgggactttccaaaatgtcgtaacaactccgccccattgacgcaaatgggcggtaggcgtgtacggtgggaggtctatataagcagagct

SEQ ID NO: 37 - DNA, 27 bp, Artificial Sequence
  Synthetic construct
ggtttagtgaaccgtcagatccgctag

SEQ ID NO: 38 - DNA, 51 bp, Artificial Sequence
  Synthetic construct
ggcggtcacaactccggaggtggaggtggacagagcccaggcccggcagcc

SEQ ID NO: 39 - protein, 17 aa, Artificial Sequence
  Synthetic construct
GGHNSGGGGGQSPGPAA

SEQ ID NO: 40 - DNA, 75 bp, Artificial Sequence
  Synthetic construct
tccggtggaggtggatccatggcttctaactttactcagttcgttctcgtcgacaatggcggaactggcgacgtg

SEQ ID NO: 41 - protein, 25 aa, Artificial Sequence
  Synthetic construct
SGGGGSMASNFTQFVLVDNGGTGDV

SEQ ID NO: 42 - DNA, 717 bp, Artificial Sequence
  Synthetic construct
atggcggtggaaggaggaatgaaatgtgtgaagttcttgctctacgtcctcctgctggccttttgcgcctgtgcagtgggactgattgccgtgggtgtcggggcacagcttgtcctgagtcagaccataatccagggggctacccctggctctctgttgccagtggtcatcatcgcagtgggtgtcttcctcttcctggtggcttttgtgggctgctgcggggcctgcaaggagaactattgtcttatgatcacgtttgccatctttctgtctcttatcatgttggtggaggtggccgcagccattgctggctatgtgtttagagataaggtgatgtcagagtttaataacaacttccggcagcagatggagaattacccgaaaaataaccacactgcttcgatcctggacaggatgcaggcagattttaagtgctgtggggctgctaactacacagattgggagaaaatcccttccatgtcgaagaaccgagtccccgactcctgctgcattaatgttactgtgggctgtgggattaatttcaacgagaaggcgatccataaggagggctgtgtggagaagattgggggctggctgaggaaaaatgtgctggtggtagctgcagcagcccttggaattgcttttgtcgaggttttgggaattgtctttgcctgctgcctcgtgaagagtatcagaagtggctacgaggtgatgtag

SEQ ID NO: 43 - protein, 238 aa, Artificial Sequence
  Synthetic construct
MAVEGGMKCVKFLLYVLLLAFCACAVGLIAVGVGAQLVLSQTIIQGATPGSLLPVVIIAVGVFLFLVAFVGCCGACKENYCLMITFAIFLSLIMLVEVAAAIAGYVFRDKVMSEFNNNFRQQMENYPKNNHTASILDRMQADFKCCGAANYTDWEKIPSMSKNRVPDSCCINVTVGCGINFNEKAIHKEGCVEKIGGWLRKNVLVVAAAALGIAFVEVLGIVFACCLVKSIRSGYEVM

SEQ ID NO: 44 - DNA, 1536 bp, Artificial Sequence
  Synthetic construct
atgaagtgccttttgtacttagcctttttattcattggggtgaattgcaagttcaccatagtttttccacacaaccaaaaaggaaactggaaaaatgttccttctaattaccattattgcccgtcaagctcagatttaaattggcataatgacttaataggcacagccatacaagtcaaaatgcccaagagtcacaaggctattcaagcagacggttggatgtgtcatgcttccaaatgggtcactacttgtgatttccgctggtatggaccgaagtatataacacagtccatccgatccttcactccatctgtagaacaatgcaaggaaagcattgaacaaacgaaacaaggaacttggctgaatccaggcttccctcctcaaagttgtggatatgcaactgtgacggatgccgaagcagtgattgtccaggtgactcctcaccatgtgctggttgatgaatacacaggagaatgggttgattcacagttcatcaacggaaaatgcagcaattacatatgccccactgtccataactctacaacctggcattctgactataaggtcaaagggctatgtgattctaacctcatttccatggacatcaccttcttctcagaggacggagagctatcatccctgggaaaggagggcacagggttcagaagtaactactttgcttatgaaactggaggcaaggcctgcaaaatgcaatactgcaagcattggggagtcagactcccatcaggtgtctggttcgagatggctgataaggatctctttgctgcagccagattccctgaatgcccagaagggtcaagtatctctgctccatctcagacctcagtggatgtaagtctaattcaggacgttgagaggatcttggattattccctctgccaagaaacctggagcaaaatcagagcgggtcttccaatctctccagtggatctcagctatcttgctcctaaaaacccaggaaccggtcctgctttcaccataatcaatggtaccctaaaatactttgagaccagatacatcagagtcgatattgctgctccaatcctctcaagaatggtcggaatgatcagtggaactaccacagaaagggaactgtgggatgactgggcaccatatgaagacgtggaaattggacccaatggagttctgaggaccagttcaggatataagtttcctttatacatgattggacatggtatgttggactccgatcttcatcttagctcaaaggctcaggtgttcgaacatcctcacattcaagacgctgcttcgcaacttcctgatgatgagagtttattttttggtgatactgggctatccaaaaatccaatcgagcttgtagaaggttggttcagtagttggaaaagctctattgcctcttttttctttatcatagggttaatcattggactattcttggttctccgagttggtatccatctttgcattaaattaaagcacaccaagaaaagacagatttatacagacatagagatgaaccgacttggaaagtaa

SEQ ID NO: 45 - protein, 511 aa, Artificial Sequence
  Synthetic construct
MKCLLYLAFLFIGVNCKFTIVFPHNQKGNWKNVPSNYHYCPSSSDLNWHNDLIGTAIQVKMPKSHKAIQADGWMCHASKWVTTCDFRWYGPKYITQSIRSFTPSVEQCKESIEQTKQGTWLNPGFPPQSCGYATVTDAEAVIVQVTPHHVLVDEYTGEWVDSQFINGKCSNYICPTVHNSTTWHSDYKVKGLCDSNLISMDITFFSEDGELSSLGKEGTGFRSNYFAYETGGKACKMQYCKHWGVRLPSGVWFEMADKDLFAAARFPECPEGSSISAPSQTSVDVSLIQDVERILDYSLCQETWSKIRAGLPISPVDLSYLAPKNPGTGPAFTIINGTLKYFETRYIRVDIAAPILSRMVGMISGTTTERELWDDWAPYEDVEIGPNGVLRTSSGYKFPLYMIGHGMLDSDLHLSSKAQVFEHPHIQDAASQLPDDESLFFGDTGLSKNPIELVEGWFSSWKSSIASFFFIIGLIIGLFLVLRVGIHLCIKLKHTKKRQIYTDIEMNRLGK

SEQ ID NO: 46 - DNA, 1494 bp, Artificial Sequence
  Synthetic construct
cgttacataacttacggtaaatggcccgcctggctgaccgcccaacgacccccgcccattgacgtcaataatgacgtatgttcccatagtaacgccaatagggactttccattgacgtcaatgggtggagtatttacggtaaactgcccacttggcagtacatcaagtgtatcatatgccaagtacgccccctattgacgtcaatgacggtaaatggcccgcctggcattatgcccagtacatgaccttatgggactttcctacttggcagtacatctacgtattagtcatcgctattaccatggtgatgcggttttggcagtacatcaatgggcgtggatagcggtttgactcacggggatttccaagtctccaccccattgacgtcaatgggagtttgttttggcaccaaaatcaacgggactttccaaaatgtcgtaacaactccgccccattgacgcaaatgggcggtaggcgtgtacggtgggaggtctatataagcagagctggtttagtgaaccgtcagatccgctagccaccatgaaatcaattcgctgtaaaaactgcaacaaactgttatttaaggcggattcctttgatcacattgaaatcaggtgtccgcgttgcaaacgtcacatcataatgctcaacgcttgtgaacaccctacggagaaacattgtgggaaaagagaaaaaatcacgcattctgacgaaaccgtgcgttatggcggtcacaactccggaggtggaggtggacagagcccaggcccggcagccatggcggtggaaggaggaatgaaatgtgtgaagttcttgctctacgtcctcctgctggccttttgcgcctgtgcagtgggactgattgccgtgggtgtcggggcacagcttgtcctgagtcagaccataatccagggggctacccctggctctctgttgccagtggtcatcatcgcagtgggtgtcttcctcttcctggtggcttttgtgggctgctgcggggcctgcaaggagaactattgtcttatgatcacgtttgccatctttctgtctcttatcatgttggtggaggtggccgcagccattgctggctatgtgtttagagataaggtgatgtcagagtttaataacaacttccggcagcagatggagaattacccgaaaaataaccacactgcttcgatcctggacaggatgcaggcagattttaagtgctgtggggctgctaactacacagattgggagaaaatcccttccatgtcgaagaaccgagtccccgactcctgctgcattaatgttactgtgggctgtgggattaatttcaacgagaaggcgatccataaggagggctgtgtggagaagattgggggctggctgaggaaaaatgtgctggtggtagctgcagcagcccttggaattgcttttgtcgaggttttgggaattgtctttgcctgctgcctcgtgaagagtatcagaagtggctacgaggtgatgtag

SEQ ID NO: 47 - protein, 317 aa, Artificial Sequence
  Synthetic construct
MKSIRCKNCNKLLFKADSFDHIEIRCPRCKRHIIMLNACEHPTEKHCGKREKITHSDETVRYGGHNSGGGGGQSPGPAAMAVEGGMKCVKFLLYVLLLAFCACAVGLIAVGVGAQLVLSQTIIQGATPGSLLPVVIIAVGVFLFLVAFVGCCGACKENYCLMITFAIFLSLIMLVEVAAAIAGYVFRDKVMSEFNNNFRQQMENYPKNNHTASILDRMQADFKCCGAANYTDWEKIPSMSKNRVPDSCCINVTVGCGINFNEKAIHKEGCVEKIGGWLRKNVLVVAAAALGIAFVEVLGIVFACCLVKSIRSGYEVM

SEQ ID NO: 48 - DNA, 1646 bp, Artificial Sequence
  Synthetic construct
gacattgattattgactagttattaatagtaatcaattacggggtcattagttcatagcccatatatggagttccgcgttacataacttacggtaaatggcccgcctggctgaccgcccaacgacccccgcccattgacgtcaataatgacgtatgttcccatagtaacgccaatagggactttccattgacgtcaatgggtggagtatttacggtaaactgcccacttggcagtacatcaagtgtatcatatgccaagtacgccccctattgacgtcaatgacggtaaatggcccgcctggcattatgcccagtacatgaccttatgggactttcctacttggcagtacatctacgtattagtcatcgctattaccatggtgatgcggttttggcagtacatcaatgggcgtggatagcggtttgactcacggggatttccaagtctccaccccattgacgtcaatgggagtttgttttggcaccaaaatcaacgggactttccaaaatgtcgtaacaactccgccccattgacgcaaatgggcggtaggcgtgtacggtgggaggtctatataagcagagctggtttagtgaaccgtcagatccgctagtcgagctcaagcttcgaattctgcagtcgacggtaccagagcccaggcccggcagccatggcggtggaaggaggaatgaaatgtgtgaagttcttgctctacgtcctcctgctggccttttgcgcctgtgcagtgggactgattgccgtgggtgtcggggcacagcttgtcctgagtcagaccataatccagggggctacccctggctctctgttgccagtggtcatcatcgcagtgggtgtcttcctcttcctggtggcttttgtgggctgctgcggggcctgcaaggagaactattgtcttatgatcacgtttgccatctttctgtctcttatcatgttggtggaggtggccgcagccattgctggctatgtgtttagagataaggtgatgtcagagtttaataacaacttccggcagcagatggagaattacccgaaaaataaccacactgcttcgatcctggacaggatgcaggcagattttaagtgctgtggggctgctaactacacagattgggagaaaatcccttccatgtcgaagaaccgagtccccgactcctgctgcattaatgttactgtgggctgtgggattaatttcaacgagaaggcgatccataaggagggctgtgtggagaagattgggggctggctgaggaaaaatgtgctggtggtagctgcagcagcccttggaattgcttttgtcgaggttttgggaattgtctttgcctgctgcctcgtgaagagtatcagaagtggctacgaggtgatgtccggtggaggtggatccatggcttctaactttactcagttcgttctcgtcgacaatggcggaactggcgacgtgatgaaatcaattcgctgtaaaaactgcaacaaactgttatttaaggcggattcctttgatcacattgaaatcaggtgtccgcgttgcaaacgtcacatcataatgctcaacgcttgtgaacaccctacggagaaacattgtgggaaaagagaaaaaatcacgcattctgacgaaaccgtgcgttattag

SEQ ID NO: 49 - protein, 325 aa, Artificial Sequence
  Synthetic construct
MAVEGGMKCVKFLLYVLLLAFCACAVGLIAVGVGAQLVLSQTIIQGATPGSLLPVVIIAVGVFLFLVAFVGCCGACKENYCLMITFAIFLSLIMLVEVAAAIAGYVFRDKVMSEFNNNFRQQMENYPKNNHTASILDRMQADFKCCGAANYTDWEKIPSMSKNRVPDSCCINVTVGCGINFNEKAIHKEGCVEKIGGWLRKNVLVVAAAALGIAFVEVLGIVFACCLVKSIRSGYEVMSGGGGSMASNFTQFVLVDNGGTGDVMKSIRCKNCNKLLFKADSFDHIEIRCPRCKRHIIMLNACEHPTEKHCGKREKITHSDETVRY

SEQ ID NO: 50 - DNA, 1755 bp, Artificial Sequence
  Synthetic construct
cgttacataacttacggtaaatggcccgcctggctgaccgcccaacgacccccgcccattgacgtcaataatgacgtatgttcccatagtaacgccaatagggactttccattgacgtcaatgggtggagtatttacggtaaactgcccacttggcagtacatcaagtgtatcatatgccaagtacgccccctattgacgtcaatgacggtaaatggcccgcctggcattatgcccagtacatgaccttatgggactttcctacttggcagtacatctacgtattagtcatcgctattaccatggtgatgcggttttggcagtacatcaatgggcgtggatagcggtttgactcacggggatttccaagtctccaccccattgacgtcaatgggagtttgttttggcaccaaaatcaacgggactttccaaaatgtcgtaacaactccgccccattgacgcaaatgggcggtaggcgtgtacggtgggaggtctatataagcagagctggtttagtgaaccgtcagatccgctagccaccatgaaatcaattcgctgtaaaaactgcaacaaactgttatttaaggcggattcctttgatcacattgaaatcaggtgtccgcgttgcaaacgtcacatcataatgctcaacgcttgtgaacaccctacggagaaacattgtgggaaaagagaaaaaatcacgcattctgacgaaaccgtgcgttatggcggtcacaactccggaggtggaggtggacagagcccaggcccggcagccatggcggtggaaggaggaatgaaatgtgtgaagttcttgctctacgtcctcctgctggccttttgcgcctgtgcagtgggactgattgccgtgggtgtcggggcacagcttgtcctgagtcagaccataatccagggggctacccctggctctctgttgccagtggtcatcatcgcagtgggtgtcttcctcttcctggtggcttttgtgggctgctgcggggcctgcaaggagaactattgtcttatgatcacgtttgccatctttctgtctcttatcatgttggtggaggtggccgcagccattgctggctatgtgtttagagataaggtgatgtcagagtttaataacaacttccggcagcagatggagaattacccgaaaaataaccacactgcttcgatcctggacaggatgcaggcagattttaagtgctgtggggctgctaactacacagattgggagaaaatcccttccatgtcgaagaaccgagtccccgactcctgctgcattaatgttactgtgggctgtgggattaatttcaacgagaaggcgatccataaggagggctgtgtggagaagattgggggctggctgaggaaaaatgtgctggtggtagctgcagcagcccttggaattgcttttgtcgaggttttgggaattgtctttgcctgctgcctcgtgaagagtatcagaagtggctacgaggtgatgtccggtggaggtggatccatggcttctaactttactcagttcgttctcgtcgacaatggcggaactggcgacgtgatgaaatcaattcgctgtaaaaactgcaacaaactgttatttaaggcggattcctttgatcacattgaaatcaggtgtccgcgttgcaaacgtcacatcataatgctcaacgcttgtgaacaccctacggagaaacattgtgggaaaagagaaaaaatcacgcattctgacgaaaccgtgcgttattag

SEQ ID NO: 51 - protein, 404 aa, Artificial Sequence
  Synthetic construct
MKSIRCKNCNKLLFKADSFDHIEIRCPRCKRHIIMLNACEHPTEKHCGKREKITHSDETVRYGGHNSGGGGGQSPGPAAMAVEGGMKCVKFLLYVLLLAFCACAVGLIAVGVGAQLVLSQTIIQGATPGSLLPVVIIAVGVFLFLVAFVGCCGACKENYCLMITFAIFLSLIMLVEVAAAIAGYVFRDKVMSEFNNNFRQQMENYPKNNHTASILDRMQADFKCCGAANYTDWEKIPSMSKNRVPDSCCINVTVGCGINFNEKAIHKEGCVEKIGGWLRKNVLVVAAAALGIAFVEVLGIVFACCLVKSIRSGYEVMSGGGGSMASNFTQFVLVDNGGTGDVMKSIRCKNCNKLLFKADSFDHIEIRCPRCKRHIIMLNACEHPTEKHCGKREKITHSDETVRY

SEQ ID NO: 52 - DNA, 25 bp, Artificial Sequence
  Synthetic construct
caccgacacagacagactacaccca

SEQ ID NO: 53 - DNA, 23 bp, Artificial Sequence
  Synthetic construct
gataaacacggcattttgccttg

SEQ ID NO: 54 - DNA, 20 bp, Artificial Sequence
  Synthetic construct
tccatttcaggtgtcgtgag

SEQ ID NO: 55 - DNA, 18 bp, Artificial Sequence
  Synthetic construct
tccagctcgaccaggatg

SEQ ID NO: 56 - DNA, 21 bp, Artificial Sequence
  Synthetic construct
gaagctatgacagaggaaacg

SEQ ID NO: 57 - DNA, 21 bp, Artificial Sequence
  Synthetic construct
agccagggctgggcataaaag

SEQ ID NO: 58 - DNA, 25 bp, Artificial Sequence
  Synthetic construct
tgggaaaatagaccaataggcagag

SEQ ID NO: 59 - DNA, 20 bp, Artificial Sequence
  Synthetic construct
ggcagctgcaggaataagag

SEQ ID NO: 60 - DNA, 19 bp, Artificial Sequence
  Synthetic construct
gctgctctttctggcattg

SEQ ID NO: 61 - DNA, 20 bp, Artificial Sequence
  Synthetic construct
tccagccattgtgttgaatc

SEQ ID NO: 62 - DNA, 22 bp, Artificial Sequence
  Synthetic construct
tcctgttgttcatcatcctagc

SEQ ID NO: 63 - DNA, 20 bp, Artificial Sequence
  Synthetic construct
tccagccattgtgttgaatc

SEQ ID NO: 64 - DNA, 20 bp, Artificial Sequence
  Synthetic construct
gtttaagggcccgccttttg

SEQ ID NO: 65 - DNA, 20 bp, Artificial Sequence
  Synthetic construct
tgtcttacctctcggtgcct

SEQ ID NO: 66 - DNA, 19 bp, Artificial Sequence
  Synthetic construct
gctgctctttctggcattg

SEQ ID NO: 67 - DNA, 23 bp, Artificial Sequence
  Synthetic construct
cagttacagttattaccgcagca

SEQ ID NO: 68 - DNA, 20 bp, Artificial Sequence
  Synthetic construct
gtctgaggtcacacagtggg

SEQ ID NO: 69 - DNA, 21 bp, Artificial Sequence
  Synthetic construct
agccctgactcatcattaccc

SEQ ID NO: 70 - DNA, 20 bp, Artificial Sequence
  Synthetic construct
aggagtaagacccctggacc

SEQ ID NO: 71 - DNA, 20 bp, Artificial Sequence
  Synthetic construct
tctcaccttgacacaagccc

SEQ ID NO: 72 - DNA, 20 bp, Artificial Sequence
  Synthetic construct
ctggcattctgggagcttca

SEQ ID NO: 73 - DNA, 20 bp, Artificial Sequence
  Synthetic construct
gagacctgtgggaagcgaaa

SEQ ID NO: 74 - DNA, 20 bp, Artificial Sequence
  Synthetic construct
gtctgaggtcacacagtggg

SEQ ID NO: 75 - DNA, 20 bp, Artificial Sequence
  Synthetic construct
ctgagagcagggaccacatc

SEQ ID NO: 76 - DNA, 23 bp, Artificial Sequence
  Synthetic construct
gcgcttgctcttcattccctggg

SEQ ID NO: 77 - DNA, 23 bp, Artificial Sequence
  Synthetic construct
gtaacggcagacttctcctcagg

SEQ ID NO: 78 - DNA, 23 bp, Artificial Sequence
  Synthetic construct
actgttgcctccggttctgaagg

SEQ ID NO: 79 - DNA, 23 bp, Artificial Sequence
  Synthetic construct
gaggacaagtcgtacaatggtgg

SEQ ID NO: 80 - DNA, 23 bp, Artificial Sequence
  Synthetic construct
gatgagataatgatgagtcaggg

SEQ ID NO: 81 - DNA, 23 bp, Artificial Sequence
  Synthetic construct
ccattgttcaatatcgtccgggg

SEQ ID NO: 82 - DNA, 23 bp, Artificial Sequence
  Synthetic construct
agccccagcaagagcacaagagg

SEQ ID NO: 83 - DNA, 27 bp, Artificial Sequence
  Synthetic construct
tatgtggctttaccaaggtcccagagt

SEQ ID NO: 84 - DNA, 27 bp, Artificial Sequence
  Synthetic construct
gtgttattacttgctactgcagagagt

SEQ ID NO: 85 - DNA, 26 bp, Artificial Sequence
  Synthetic construct
acacagacagactacacccagggaat

SEQ ID NO: 86 - DNA, 24 bp, Artificial Sequence
  Synthetic construct
accggcgcttgctcttcattccct

SEQ ID NO: 87 - DNA, 24 bp, Artificial Sequence
  Synthetic construct
accggtaacggcagacttctccac

SEQ ID NO: 88 - DNA, 24 bp, Artificial Sequence
  Synthetic construct
accgactgttgcctccggttctga

SEQ ID NO: 89 - DNA, 24 bp, Artificial Sequence
  Synthetic construct
accggaggacaagtcgtacaatgg

SEQ ID NO: 90 - DNA, 24 bp, Artificial Sequence
  Synthetic construct
accggatgagataatgatgagtca

SEQ ID NO: 91 - DNA, 24 bp, Artificial Sequence
  Synthetic construct
accgccattgttcaatatcgtccg

SEQ ID NO: 92 - DNA, 24 bp, Artificial Sequence
  Synthetic construct
accgagccccagcaagagcacaag

SEQ ID NO: 93 - DNA, 26 bp, Artificial Sequence
  Synthetic construct
caccgtatgtggctttaccaaggtcc

SEQ ID NO: 94 - DNA, 25 bp, Artificial Sequence
  Synthetic construct
caccgtgttattacttgctactgca

SEQ ID NO: 95 - DNA, 25 bp, Artificial Sequence
  Synthetic construct
caccgacacagacagactacaccca

SEQ ID NO: 96 - DNA, 24 bp, Artificial Sequence
  Synthetic construct
aaacagggaatgaagagcaagcgc

SEQ ID NO: 97 - DNA, 24 bp, Artificial Sequence
  Synthetic construct
aaacgtggagaagtctgccgttac

SEQ ID NO: 98 - DNA, 24 bp, Artificial Sequence
  Synthetic construct
aaactcagaaccggaggcaacagt

SEQ ID NO: 99 - DNA, 24 bp, Artificial Sequence
  Synthetic construct
aaacccattgtacgacttgtcctc

SEQ ID NO: 100 - DNA, 24 bp, Artificial Sequence
  Synthetic construct
aaactgactcatcattatctcatc

SEQ ID NO: 101 - DNA, 24 bp, Artificial Sequence
  Synthetic construct
aaaccggacgatattgaacaatgg

SEQ ID NO: 102 - DNA, 24 bp, Artificial Sequence
  Synthetic construct
aaaccttgtgctcttgctggggct

SEQ ID NO: 103 - DNA, 26 bp, Artificial Sequence
  Synthetic construct
aaacggaccttggtaaagccacatac

SEQ ID NO: 104 - DNA, 25 bp, Artificial Sequence
  Synthetic construct
aaactgcagtagcaagtaataacac

SEQ ID NO: 105 - DNA, 25 bp, Artificial Sequence
  Synthetic construct
aaactgggtgtagtctgtctgtgtc

SEQ ID NO: 106 - DNA, 6 bp, Artificial Sequence
  Synthetic construct
  misc_feature (1)..(2): n is a, c, g, or t
nngrrt

SEQ ID NO: 107 - DNA, 6 bp, Artificial Sequence
  Synthetic construct
  misc_feature (1)..(2): n is a, c, g, or t
  misc_feature (6)..(6): n is a, c, g, or t
nngrrn

SEQ ID NO: 108 - RNA, 6 nt, Artificial Sequence
  Synthetic construct
aauaaa

SEQ ID NO: 109 - DNA, 19 bp, Artificial Sequence
  Synthetic construct
ttgggggctggctgaggaa

SEQ ID NO: 110 - DNA, 42 bp, Artificial Sequence
  Synthetic construct
ccatggatccacctccaccggacatcacctcgtagccacttc

SEQ ID NO: 111 - DNA, 42 bp, Artificial Sequence
  Synthetic construct
gaagtggctacgaggtgatgtccggtggaggtggatccatgg

SEQ ID NO: 112 - DNA, 44 bp, Artificial Sequence
  Synthetic construct
tagatccggtggatcagatctctaataacgcacggtttcgtcag

SEQ ID NO: 113 - DNA, 44 bp, Artificial Sequence; identical to SEQ ID NO: 112
  Synthetic construct

SEQ ID NO: 114 - DNA, 60 bp, Artificial Sequence
  Synthetic construct
cgggcctgggctctgtccacctccacctccggagttgtgaccgccataacgcacggtttc

SEQ ID NO: 115 - protein, 17 aa, Artificial sequence
  Synthetic construct
GGHNSGGGGGQSPGPAA

SEQ ID NO: 116 - protein, 25 aa, Artificial sequence
  Synthetic construct
SGGGGSMASNFTQFVLVDNGGTGDV